European Patent Specification EP 3 861 854 B1, published January 22, 2025. Title: Immunodeficient mouse. Applicant: Central Institute for Experimental Animals. The sequence listing filed with the application follows.

SEQUENCE LISTING (13 sequences)

SEQ ID NO: 1 - DNA, 21 bp, Artificial
  Inventor: Takahashi, Takeshi; Katano, Ikumi
  Fcer1g primer 1
ctcgtgctttacggtatcgcc

SEQ ID NO: 2 - DNA, 22 bp, Artificial
  Fcer1g primer2
cctactctactgtcgactcaag

SEQ ID NO: 3 - DNA, 21 bp, Artificial
  Fcer1g primer3
ggctggctatagctgcctttc

SEQ ID NO: 4 - DNA, 21 bp, Artificial
  Fcgr2b primer1
ctcgtgctttacggtatcgcc

SEQ ID NO: 5 - DNA, 21 bp, Artificial
  Fcgr2b primer2
aaactcgaccccccgtggatc

SEQ ID NO: 6 - DNA, 24 bp, Artificial
  Fcgr2b primer3
ttgactgtggccttaaacgtgtag

SEQ ID NO: 7 - DNA, 23 bp, Artificial
  IL-2rg primer1
ctgctcagaatgcctccaattcc

SEQ ID NO: 8 - DNA, 26 bp, Artificial
  IL-2rg primer2
cctccgtgcaatccatcttgttcaat

SEQ ID NO: 9 - DNA, 24 bp, Artificial
  IL-2rg primer3
gatccagattgccaaggtgagtag

SEQ ID NO: 10 - DNA, 20 bp, Artificial
  scid primer1
gctagagagctgttccagtt

SEQ ID NO: 11 - DNA, 21 bp, Artificial
  scid primer2
tttgaacacacactgattctg

SEQ ID NO: 12 - DNA, 9 bp, Artificial
  scid primer3
acgctaagc

SEQ ID NO: 13 - DNA, 9 bp, Artificial
  scid primer4
cgctatgct